European Patent Application EP 4 501 943 A1, published February 5, 2025. Title: Peptide, Peptide Complex Having Activity of Anti-Diabetes and Uses Thereof. Applicant: CAREGEN CO., LTD. The sequence listing filed with the application follows.

SEQUENCE LISTING (28 sequences)

SEQ ID NO: 1 - protein, 5 aa, Artificial Sequence
  Peptide
LKTRN

SEQ ID NO: 2 - protein, 9 aa, Artificial Sequence
  Peptide
KGSATGWMA

SEQ ID NO: 3 - DNA, 20 bp, Artificial Sequence
  TNF-alpha Forward primer
cgtcagccgatttgctatct

SEQ ID NO: 4 - DNA, 20 bp, Artificial Sequence
  TNF-alpha Reverse primer
cggactccgcaaagtctaag

SEQ ID NO: 5 - DNA, 25 bp, Artificial Sequence
  mTOR forward primer
ttgaggtcgctatgaccagagagaa

SEQ ID NO: 6 - DNA, 25 bp, Artificial Sequence
  mTOR reverse primer
ttaccagaagggacaccagccaatg

SEQ ID NO: 7 - DNA, 21 bp, Artificial Sequence
  p70S6K forward primer
ggagcctgggagccctgatgt

SEQ ID NO: 8 - DNA, 22 bp, Artificial Sequence
  p70S6K reverse primer
gaagccctctttgatgctgtcc

SEQ ID NO: 9 - DNA, 20 bp, Artificial Sequence
  GAPDH forward primer
gtgatggcatggactgtggt

SEQ ID NO: 10 - DNA, 20 bp, Artificial Sequence
  GAPDH reverse primer
ggagccaaaagggtcatcat

SEQ ID NO: 11 - DNA, 20 bp, Artificial Sequence
  Leptin forward primer
ggatcaggttttgtggtgct

SEQ ID NO: 12 - DNA, 20 bp, Artificial Sequence
  Leptin reverse primer
ttgtggcccataaagtcctc

SEQ ID NO: 13 - DNA, 20 bp, Artificial Sequence
  Adiponectin forward primer
tcctgctttggtccctccac

SEQ ID NO: 14 - DNA, 20 bp, Artificial Sequence
  Adiponectin reverse primer
tctccagccccacactgaac

SEQ ID NO: 15 - DNA, 20 bp, Artificial Sequence
  IRS-1 forward primer
gccaatcttcatccagttgc

SEQ ID NO: 16 - DNA, 20 bp, Artificial Sequence
  IRS-1 reverse primer
catcgtgaagaaggcatagg

SEQ ID NO: 17 - DNA, 20 bp, Artificial Sequence
  TNF-alpha forward primer
atgagcacggaaagcatgat

SEQ ID NO: 18 - DNA, 20 bp, Artificial Sequence
  TNF-alpha reverse primer
ctcttgatggcagagaggag

SEQ ID NO: 19 - DNA, 23 bp, Artificial Sequence
  PGC-1 forward primer
agtctgtatggagtgacatcgag

SEQ ID NO: 20 - DNA, 20 bp, Artificial Sequence
  PGC-1 reverse primer
ggcaatccgtcttcatccac

SEQ ID NO: 21 - DNA, 19 bp, Artificial Sequence
  ACOX-1 forward primer
ccgccgagagatcgagaac

SEQ ID NO: 22 - DNA, 20 bp, Artificial Sequence
  ACOX-1 reverse primer
cagttgcctggtgaagcaag

SEQ ID NO: 23 - DNA, 20 bp, Artificial Sequence
  PPAR-alpha forward primer
aagggcttctttcggcgaac

SEQ ID NO: 24 - DNA, 27 bp, Artificial Sequence
  PPAR-alpha reverse primer
tgaccttgttcatgttgaagttcttca

SEQ ID NO: 25 - DNA, 20 bp, Artificial Sequence
  CTP-1alpha forward primer
cctccagttggcttatcgtg

SEQ ID NO: 26 - DNA, 20 bp, Artificial Sequence
  CTP-1alpha reverse primer
ttcttcgtctggctggacat

SEQ ID NO: 27 - DNA, 20 bp, Artificial Sequence
  GLUT4 forward primer
actaagagcaccgagaccaa

SEQ ID NO: 28 - DNA, 20 bp, Artificial Sequence
  GLUT4 reverse primer
ctgcccgaaagagtctaaag